European Patent Application EP 4 800 038 A1, published September 2, 2026. Title: 靶向CD19的嵌合抗原受体的治疗用途. Applicant: 上海先博生物科技有限公司. The sequence listing filed with the application follows.

SEQUENCE LISTING (26 sequences)

SEQ ID NO: 1 - protein, 119 aa, synthetic construct
QVQLQQPGAELVVPGTSVKLSCKASGYTFTNYWMHWVKQRPGQGLEWIGEIDPSDNYANYNQEFQGKATLTVDKSSSTAYMQLSSLTSDDSAVYYCARHDGYFGALDYWGQGTSVTVSS

SEQ ID NO: 2 - protein, 110 aa, synthetic construct
EIVLTQSPTTMAASPGEKITITCSASSSISSNYLHWYQQKPGFSPKFLIYRTSNLASGVPARFSGSGSGTSYSLTIGTMEAEDVATYYCQQASSIPRMFTFGSGTKLEIK

SEQ ID NO: 3 - protein, 120 aa, synthetic construct
EVKLQESGPGLVAPSQSLSVTCTVSGVSLPDYGVSWIRQPPRKGLEWLGVIWGSETTYYNSALKSRLTIIKDNSKSQVFLKMNSLQTDDTAIYYCAKHYYYGGSYAMDYWGQGTSVTVSS

SEQ ID NO: 4 - protein, 107 aa, synthetic construct
DIQMTQTTSSLSASLGDRVTISCRASQDISKYLNWYQQKPDGTVKLLIYHTSRLHSGVPSRFSGSGSGTDYSLTISNLEQEDIATYFCQQGNTLPYTFGGGTKLEIT

SEQ ID NO: 5 - protein, 5 aa, synthetic construct
NYWMH

SEQ ID NO: 6 - protein, 17 aa, synthetic construct
EIDPSDNYANYNQEFQG

SEQ ID NO: 7 - protein, 10 aa, synthetic construct
HDGYFGALDY

SEQ ID NO: 8 - protein, 12 aa, synthetic construct
SASSSISSNYLH

SEQ ID NO: 9 - protein, 7 aa, synthetic construct
RTSNLAS

SEQ ID NO: 10 - protein, 11 aa, synthetic construct
QQASSIPRMFT

SEQ ID NO: 11 - protein, 5 aa, synthetic construct
DYGVS

SEQ ID NO: 12 - protein, 16 aa, synthetic construct
VIWGSETTYYNSALKS

SEQ ID NO: 13 - protein, 12 aa, synthetic construct
HYYYGGSYAMDY

SEQ ID NO: 14 - protein, 11 aa, synthetic construct
RASQDISKYLN

SEQ ID NO: 15 - protein, 7 aa, synthetic construct
HTSRLHS

SEQ ID NO: 16 - protein, 9 aa, synthetic construct
QQGNTLPYT

SEQ ID NO: 17 - protein, 110 aa, synthetic construct
EIVLTQSPATLSLSPGERATLSCSASSSISSNYLHWYQQKPGQAPRFLIYRTSNLASGIPARFSGSGSGTDFTLTISSLEPEDFAVYYCQQASSIPRMFTFGQGTKLEIK

SEQ ID NO: 18 - protein, 110 aa, synthetic construct
EIVLTQSPDFQSVTPKEKVTITCSASSSISSNYLHWYQQKPDQSPKFLIYRTSNLASGVPSRFSGSGSGTDFTLTINSLEAEDAATYYCQQASSIPRMFTFGQGTKLEIK

SEQ ID NO: 19 - protein, 119 aa, synthetic construct
EVQLVQSGAEVKKPGASVKVSCKASGYTFTNYWMHWVRQRPGQGLEWMGEIDPSDNYANYNQEFQGRVTITVDKSASTAYMELSSLRSEDTAVYYCARHDGYFGALDYWGQGTTVTVSS

SEQ ID NO: 20 - protein, 119 aa, synthetic construct
EVQLQQSGAEVKKPGASVKVSCKASGYTFTNYWMHWVRQRPGQGLEWMGEIDPSDNYANYNQEFQGRVTITVDKSASTAYMELSSLRSEDTAVYYCARHDGYFGALDYWGQGTTVTVSS

SEQ ID NO: 21 - protein, 107 aa, synthetic construct
DIQMTQSPSSLSASVGDRVTITCRASQDISKYLNWYQQKPGGAVKLLIYHTSRLHSGVPSRFSGSGSGTDYTLTISSLQPEDFATYYCQQGNTLPYTFGGGTKVEIK

SEQ ID NO: 22 - protein, 120 aa, synthetic construct
EVTLKESGPVLVKPTETLTLTCTVSGFSLSDYGVSWIRQPPGKALEWLAVIWGSETTYYNSALKSRLTISKDTSKSQVVLTMTNMDPVDTATYYCAKHYYYGGSYAMDYWGQGTTVTVSS

SEQ ID NO: 23 - protein, 688 aa, synthetic construct
MALPVTALLLPLALLLHAARPLEEIVLTQSPATLSLSPGERATLSCSASSSISSNYLHWYQQKPGQAPRFLIYRTSNLASGIPARFSGSGSGTDFTLTISSLEPEDFAVYYCQQASSIPRMFTFGQGTKLEIKGSTSGSGKPGSGEGSTKGEVQLQQSGAEVKKPGASVKVSCKASGYTFTNYWMHWVRQRPGQGLEWMGEIDPSDNYANYNQEFQGRVTITVDKSASTAYMELSSLRSEDTAVYYCARHDGYFGALDYWGQGTTVTVSSGSFVPVFLPAKRTTTPAPRPPTPAPTIASQPLSLRPEACRPAAGGAVHTRGLDFACDIYIWAPLAGTCGVLLLSLVITLYCRSKRSRLLHSDYMNMTPRRPGPTRKHYQPYAPPRDFAAYRSRVKFSRSADAPAYQQGQNQLYNELNLGRREEYDVLDKRRGRDPEMGGKPRRKNPQEGLYNELQKDKMAEAYSEIGMKGERRRGKGHDGLYQGLSTATKDTYDALHMQALPPRGSGATNFSLLKQAGDVEENPGPMRISKPHLRSISIQCYLCLLLNSHFLTEAGIHVFILGCFSAGLPKTEANWVNVISDLKKIEDLIQSMHIDATLYTESDVHPSCKVTAMKCFLLELQVISLESGDASIHDTVENLIILANNSLSSNGNVTESGCKECEELEEKNIKEFLQSFVHIVQMFINTS

SEQ ID NO: 24 - protein, 688 aa, synthetic construct
MALPVTALLLPLALLLHAARPLEEIVLTQSPDFQSVTPKEKVTITCSASSSISSNYLHWYQQKPDQSPKFLIYRTSNLASGVPSRFSGSGSGTDFTLTINSLEAEDAATYYCQQASSIPRMFTFGQGTKLEIKGSTSGSGKPGSGEGSTKGEVQLVQSGAEVKKPGASVKVSCKASGYTFTNYWMHWVRQRPGQGLEWMGEIDPSDNYANYNQEFQGRVTITVDKSASTAYMELSSLRSEDTAVYYCARHDGYFGALDYWGQGTTVTVSSGSFVPVFLPAKRTTTPAPRPPTPAPTIASQPLSLRPEACRPAAGGAVHTRGLDFACDIYIWAPLAGTCGVLLLSLVITLYCRSKRSRLLHSDYMNMTPRRPGPTRKHYQPYAPPRDFAAYRSRVKFSRSADAPAYQQGQNQLYNELNLGRREEYDVLDKRRGRDPEMGGKPRRKNPQEGLYNELQKDKMAEAYSEIGMKGERRRGKGHDGLYQGLSTATKDTYDALHMQALPPRGSGATNFSLLKQAGDVEENPGPMRISKPHLRSISIQCYLCLLLNSHFLTEAGIHVFILGCFSAGLPKTEANWVNVISDLKKIEDLIQSMHIDATLYTESDVHPSCKVTAMKCFLLELQVISLESGDASIHDTVENLIILANNSLSSNGNVTESGCKECEELEEKNIKEFLQSFVHIVQMFINTS

SEQ ID NO: 25 - protein, 686 aa, synthetic construct
MALPVTALLLPLALLLHAARPLEDIQMTQSPSSLSASVGDRVTITCRASQDISKYLNWYQQKPGGAVKLLIYHTSRLHSGVPSRFSGSGSGTDYTLTISSLQPEDFATYYCQQGNTLPYTFGGGTKVEIKGSTSGSGKPGSGEGSTKGEVTLKESGPVLVKPTETLTLTCTVSGFSLSDYGVSWIRQPPGKALEWLAVIWGSETTYYNSALKSRLTISKDTSKSQVVLTMTNMDPVDTATYYCAKHYYYGGSYAMDYWGQGTTVTVSSGSFVPVFLPAKRTTTPAPRPPTPAPTIASQPLSLRPEACRPAAGGAVHTRGLDFACDIYIWAPLAGTCGVLLLSLVITLYCRSKRSRLLHSDYMNMTPRRPGPTRKHYQPYAPPRDFAAYRSRVKFSRSADAPAYQQGQNQLYNELNLGRREEYDVLDKRRGRDPEMGGKPRRKNPQEGLYNELQKDKMAEAYSEIGMKGERRRGKGHDGLYQGLSTATKDTYDALHMQALPPRGSGATNFSLLKQAGDVEENPGPMRISKPHLRSISIQCYLCLLLNSHFLTEAGIHVFILGCFSAGLPKTEANWVNVISDLKKIEDLIQSMHIDATLYTESDVHPSCKVTAMKCFLLELQVISLESGDASIHDTVENLIILANNSLSSNGNVTESGCKECEELEEKNIKEFLQSFVHIVQMFINTS

SEQ ID NO: 26 - protein, 686 aa, synthetic construct
MALPVTALLLPLALLLHAARPLEDIQMTQTTSSLSASLGDRVTISCRASQDISKYLNWYQQKPDGTVKLLIYHTSRLHSGVPSRFSGSGSGTDYSLTISNLEQEDIATYFCQQGNTLPYTFGGGTKLEITGSTSGSGKPGSGEGSTKGEVKLQESGPGLVAPSQSLSVTCTVSGVSLPDYGVSWIRQPPRKGLEWLGVIWGSETTYYNSALKSRLTIIKDNSKSQVFLKMNSLQTDDTAIYYCAKHYYYGGSYAMDYWGQGTSVTVSSGSFVPVFLPAKRTTTPAPRPPTPAPTIASQPLSLRPEACRPAAGGAVHTRGLDFACDIYIWAPLAGTCGVLLLSLVITLYCRSKRSRLLHSDYMNMTPRRPGPTRKHYQPYAPPRDFAAYRSRVKFSRSADAPAYQQGQNQLYNELNLGRREEYDVLDKRRGRDPEMGGKPRRKNPQEGLYNELQKDKMAEAYSEIGMKGERRRGKGHDGLYQGLSTATKDTYDALHMQALPPRGSGATNFSLLKQAGDVEENPGPMRISKPHLRSISIQCYLCLLLNSHFLTEAGIHVFILGCFSAGLPKTEANWVNVISDLKKIEDLIQSMHIDATLYTESDVHPSCKVTAMKCFLLELQVISLESGDASIHDTVENLIILANNSLSSNGNVTESGCKECEELEEKNIKEFLQSFVHIVQMFINTS